European Patent Specification EP 3 871 680 B1, published March 20, 2024. Title: C5 EXPRESSION INHIBITING DOUBLE-STRANDED RIBONUCLEIC ACID. Applicant: Eisai R&D Management Co., Ltd. The sequence listing filed with the application follows.

SEQUENCE LISTING (172 sequences)

SEQ ID NO: 1 - RNA, 21 nt, Artificial Sequence
  synthesized siRNA sense sequence
  misc_feature (4)..(4): cm
  misc_feature (10)..(10): um
  misc_feature (12)..(13): um
  misc_feature (14)..(14): cm
  misc_feature (20)..(21): n=deoxythymidine
  misc_feature (20)..(21): phosphorothioate bond
aggcaaagguguucaaagann

SEQ ID NO: 2 - RNA, 21 nt, Artificial Sequence
  synthesized siRNA antisense sequence
  misc_feature (9)..(9): cm
  misc_feature (20)..(21): n=deoxythymidine
  misc_feature (20)..(21): phosphorothioate bond
ucuuugaacaccuuugccunn

SEQ ID NO: 3 - RNA, 21 nt, Artificial Sequence
  synthesized siRNA sense sequence
  misc_feature (1)..(1): cm
  misc_feature (2)..(2): um
  misc_feature (4)..(4): um
  misc_feature (5)..(5): cm
  misc_feature (6)..(7): um
  misc_feature (10)..(10): cm
  misc_feature (11)..(13): um
  misc_feature (14)..(14): cm
  misc_feature (16)..(16): um
  misc_feature (20)..(21): n=deoxythymidine
  misc_feature (20)..(21): phosphorothioate bond
cugucuuaacuuucauagann

SEQ ID NO: 4 - RNA, 21 nt, Artificial Sequence
  synthesized siRNA antisense sequence
  misc_feature (3)..(3): um
  misc_feature (12)..(12): um
  misc_feature (17)..(17): cm
  misc_feature (20)..(21): n=deoxythymidine
  misc_feature (20)..(21): phosphorothioate bond
ucuaugaaaguuaagacagnn

SEQ ID NO: 5 - RNA, 21 nt, Artificial Sequence
  synthesized siRNA sense sequence
  misc_feature (1)..(1): um
  misc_feature (4)..(4): cm
  misc_feature (6)..(6): um
  misc_feature (8)..(8): um
  misc_feature (10)..(11): cm
  misc_feature (14)..(14): cm
  misc_feature (15)..(15): um
  misc_feature (17)..(17): cm
  misc_feature (20)..(21): n=deoxythymidine
  misc_feature (20)..(21): phosphorothioate bond
uagcaugugccagcuacaann

SEQ ID NO: 6 - RNA, 21 nt, Artificial Sequence
  synthesized siRNA antisense sequence
  misc_feature (4)..(4): um
  misc_feature (11)..(11): cm
  misc_feature (13)..(13): cm
  misc_feature (18)..(18): um
  misc_feature (20)..(21): n=deoxythymidine
  misc_feature (20)..(21): phosphorothioate bond
uuguagcuggcacaugcuann

SEQ ID NO: 7 - RNA, 21 nt, Artificial Sequence
  synthesized siRNA sense sequence
  misc_feature (1)..(1): cm
  misc_feature (2)..(2): um
  misc_feature (4)..(4): um
  misc_feature (7)..(8): um
  misc_feature (13)..(14): um
  misc_feature (20)..(21): n=deoxythymidine
  misc_feature (20)..(21): phosphorothioate bond
cugugauuggaauuagaaann

SEQ ID NO: 8 - RNA, 21 nt, Artificial Sequence
  synthesized siRNA antisense sequence
  misc_feature (5)..(5): um
  misc_feature (11)..(11): cm
  misc_feature (15)..(15): cm
  misc_feature (17)..(17): cm
  misc_feature (20)..(21): n=deoxythymidine
  misc_feature (20)..(21): phosphorothioate bond
uuucuaauuccaaucacagnn

SEQ ID NO: 9 - RNA, 21 nt, Artificial Sequence
  synthesized siRNA sense sequence
  misc_feature (5)..(5): cm
  misc_feature (11)..(11): um
  misc_feature (13)..(14): um
  misc_feature (15)..(15): cm
  misc_feature (20)..(21): n=deoxythymidine
  misc_feature (20)..(21): phosphorothioate bond
aaggcaaagguguucaaagnn

SEQ ID NO: 10 - RNA, 21 nt, Artificial Sequence
  synthesized siRNA antisense sequence
  misc_feature (8)..(8): cm
  misc_feature (20)..(21): n=deoxythymidine
  misc_feature (20)..(21): phosphorothioate bond
cuuugaacaccuuugccuunn

SEQ ID NO: 11 - RNA, 21 nt, Artificial Sequence
  synthesized siRNA sense sequence
  misc_feature (9)..(9): cm
  misc_feature (10)..(10): um
  misc_feature (12)..(14): um
  misc_feature (16)..(16): cm
  misc_feature (19)..(19): cm
  misc_feature (20)..(21): n=deoxythymidine
  misc_feature (20)..(21): phosphorothioate bond
gaaaggaacuguuuacaacnn

SEQ ID NO: 12 - RNA, 21 nt, Artificial Sequence
  synthesized siRNA antisense sequence
  misc_feature (5)..(5): um
  misc_feature (9)..(9): cm
  misc_feature (20)..(21): n=deoxythymidine
  misc_feature (20)..(21): phosphorothioate bond
guuguaaacaguuccuuucnn

SEQ ID NO: 13 - RNA, 21 nt, Artificial Sequence
  synthesized siRNA sense sequence
  misc_feature (1)..(1): um
  misc_feature (4)..(4): um
  misc_feature (6)..(6): um
  misc_feature (8)..(8): um
  misc_feature (10)..(10): um
  misc_feature (12)..(13): um
  misc_feature (15)..(15): cm
  misc_feature (16)..(16): um
  misc_feature (19)..(19): um
  misc_feature (20)..(21): n=deoxythymidine
  misc_feature (20)..(21): phosphorothioate bond
ugguauauguguugcugaunn

SEQ ID NO: 14 - RNA, 21 nt, Artificial Sequence
  synthesized siRNA antisense sequence
  misc_feature (3)..(3): cm
  misc_feature (6)..(6): cm
  misc_feature (9)..(9): cm
  misc_feature (11)..(11): cm
  misc_feature (13)..(13): um
  misc_feature (15)..(15): um
  misc_feature (18)..(18): cm
  misc_feature (20)..(21): n=deoxythymidine
  misc_feature (20)..(21): phosphorothioate bond
aucagcaacacauauaccann

SEQ ID NO: 15 - RNA, 21 nt, Artificial Sequence
  synthesized siRNA sense sequence
  misc_feature (2)..(2): cm
  misc_feature (3)..(3): um
  misc_feature (5)..(5): um
  misc_feature (6)..(6): cm
  misc_feature (7)..(8): um
  misc_feature (11)..(11): cm
  misc_feature (12)..(14): um
  misc_feature (15)..(15): cm
  misc_feature (17)..(17): um
  misc_feature (20)..(21): n=deoxythymidine
  misc_feature (20)..(21): phosphorothioate bond
acugucuuaacuuucauagnn

SEQ ID NO: 16 - RNA, 21 nt, Artificial Sequence
  synthesized siRNA antisense sequence
  misc_feature (2)..(2): um
  misc_feature (11)..(11): um
  misc_feature (16)..(16): cm
  misc_feature (20)..(21): n=deoxythymidine
  misc_feature (20)..(21): phosphorothioate bond
cuaugaaaguuaagacagunn

SEQ ID NO: 17 - RNA, 21 nt, Artificial Sequence
  synthesized siRNA sense sequence
  misc_feature (2)..(2): um
  misc_feature (4)..(5): cm
  misc_feature (8)..(8): cm
  misc_feature (9)..(9): um
  misc_feature (11)..(11): cm
  misc_feature (15)..(17): cm
  misc_feature (20)..(21): n=deoxythymidine
  misc_feature (20)..(21): phosphorothioate bond
gugccagcuacaagcccagnn

SEQ ID NO: 18 - RNA, 21 nt, Artificial Sequence
  synthesized siRNA antisense sequence
  misc_feature (10)..(10): um
  misc_feature (17)..(17): cm
  misc_feature (20)..(21): n=deoxythymidine
  misc_feature (20)..(21): phosphorothioate bond
cugggcuuguagcuggcacnn

SEQ ID NO: 19 - RNA, 21 nt, Artificial Sequence
  synthesized siRNA sense sequence
  misc_feature (7)..(7): cm
  misc_feature (8)..(8): um
  misc_feature (10)..(12): um
  misc_feature (14)..(14): cm
  misc_feature (17)..(17): cm
  misc_feature (18)..(18): um
  misc_feature (20)..(21): n=deoxythymidine
  misc_feature (20)..(21): phosphorothioate bond
aaggaacuguuuacaacuann

SEQ ID NO: 20 - RNA, 21 nt, Artificial Sequence
  synthesized siRNA antisense sequence
  misc_feature (1)..(1): um
  misc_feature (7)..(7): um
  misc_feature (11)..(11): cm
  misc_feature (20)..(21): n=deoxythymidine
  misc_feature (20)..(21): phosphorothioate bond
uaguuguaaacaguuccuunn

SEQ ID NO: 21 - RNA, 21 nt, Artificial Sequence
  synthesized siRNA sense sequence
  misc_feature (1)..(1): um
  misc_feature (2)..(3): cm
  misc_feature (4)..(4): um
  misc_feature (5)..(5): cm
  misc_feature (6)..(6): um
  misc_feature (12)..(13): um
  misc_feature (16)..(17): cm
  misc_feature (18)..(19): um
  misc_feature (20)..(21): n=deoxythymidine
  misc_feature (20)..(21): phosphorothioate bond
uccucuggaaauuggccuunn

SEQ ID NO: 22 - RNA, 21 nt, Artificial Sequence
  synthesized siRNA antisense sequence
  misc_feature (6)..(6): cm
  misc_feature (13)..(13): cm
  misc_feature (20)..(21): n=deoxythymidine
  misc_feature (20)..(21): phosphorothioate bond
aaggccaauuuccagaggann

SEQ ID NO: 23 - RNA, 21 nt, Artificial Sequence
  synthesized siRNA sense sequence
  misc_feature (1)..(2): um
  misc_feature (11)..(11): cm
  misc_feature (12)..(12): um
  misc_feature (14)..(16): um
  misc_feature (18)..(18): cm
  misc_feature (20)..(21): n=deoxythymidine
  misc_feature (20)..(21): phosphorothioate bond
uugaaaggaacuguuuacann

SEQ ID NO: 24 - RNA, 21 nt, Artificial Sequence
  synthesized siRNA antisense sequence
  misc_feature (3)..(3): um
  misc_feature (7)..(7): cm
  misc_feature (17)..(17): cm
  misc_feature (20)..(21): n=deoxythymidine
  misc_feature (20)..(21): phosphorothioate bond
uguaaacaguuccuuucaann

SEQ ID NO: 25 - RNA, 21 nt, Artificial Sequence
  synthesized siRNA sense sequence
  misc_feature (8)..(8): cm
  misc_feature (9)..(9): um
  misc_feature (11)..(13): um
  misc_feature (15)..(15): cm
  misc_feature (18)..(18): cm
  misc_feature (19)..(19): um
  misc_feature (20)..(21): n=deoxythymidine
  misc_feature (20)..(21): phosphorothioate bond
aaaggaacuguuuacaacunn

SEQ ID NO: 26 - RNA, 21 nt, Artificial Sequence
  synthesized siRNA antisense sequence
  misc_feature (6)..(6): um
  misc_feature (10)..(10): cm
  misc_feature (20)..(21): n=deoxythymidine
  misc_feature (20)..(21): phosphorothioate bond
aguuguaaacaguuccuuunn

SEQ ID NO: 27 - RNA, 21 nt, Artificial Sequence
  synthesized siRNA sense sequence
  misc_feature (6)..(6): cm
  misc_feature (7)..(7): um
  misc_feature (9)..(11): um
  misc_feature (13)..(13): cm
  misc_feature (16)..(16): cm
  misc_feature (17)..(17): um
  misc_feature (19)..(19): um
  misc_feature (20)..(21): n=deoxythymidine
  misc_feature (20)..(21): phosphorothioate bond
aggaacuguuuacaacuaunn

SEQ ID NO: 28 - RNA, 21 nt, Artificial Sequence
  synthesized siRNA antisense sequence
  misc_feature (2)..(2): um
  misc_feature (8)..(8): um
  misc_feature (12)..(12): cm
  misc_feature (20)..(21): n=deoxythymidine
  misc_feature (20)..(21): phosphorothioate bond
auaguuguaaacaguuccunn

SEQ ID NO: 29 - RNA, 21 nt, Artificial Sequence
  synthesized siRNA sense sequence
  misc_feature (1)..(1): um
  misc_feature (3)..(3): cm
  misc_feature (5)..(5): cm
  misc_feature (6)..(6): um
  misc_feature (11)..(11): cm
  misc_feature (13)..(15): um
  misc_feature (18)..(18): um
  misc_feature (20)..(21): n=deoxythymidine
  misc_feature (20)..(21): phosphorothioate bond
uacacugaagcauuugaugnn

SEQ ID NO: 30 - RNA, 21 nt, Artificial Sequence
  synthesized siRNA antisense sequence
  misc_feature (1)..(1): cm
  misc_feature (4)..(4): cm
  misc_feature (13)..(13): cm
  misc_feature (18)..(18): um
  misc_feature (20)..(21): n=deoxythymidine
  misc_feature (20)..(21): phosphorothioate bond
caucaaaugcuucaguguann

SEQ ID NO: 31 - RNA, 21 nt, Artificial Sequence
  synthesized siRNA sense sequence
  misc_feature (1)..(1): cm
  misc_feature (3)..(3): cm
  misc_feature (4)..(4): um
  misc_feature (9)..(9): cm
  misc_feature (11)..(13): um
  misc_feature (16)..(16): um
  misc_feature (18)..(18): cm
  misc_feature (20)..(21): n=deoxythymidine
  misc_feature (20)..(21): phosphorothioate bond
cacugaagcauuugaugcann

SEQ ID NO: 32 - RNA, 21 nt, Artificial Sequence
  synthesized siRNA antisense sequence
  misc_feature (3)..(3): cm
  misc_feature (6)..(6): cm
  misc_feature (15)..(15): cm
  misc_feature (20)..(21): n=deoxythymidine
  misc_feature (20)..(21): phosphorothioate bond
ugcaucaaaugcuucagugnn

SEQ ID NO: 33 - RNA, 21 nt, Artificial Sequence
  synthesized siRNA sense sequence
  misc_feature (1)..(1): cm
  misc_feature (2)..(2): um
  misc_feature (7)..(7): cm
  misc_feature (9)..(11): um
  misc_feature (14)..(14): um
  misc_feature (16)..(16): cm
  misc_feature (19)..(19): cm
  misc_feature (20)..(21): n=deoxythymidine
  misc_feature (20)..(21): phosphorothioate bond
cugaagcauuugaugcaacnn

SEQ ID NO: 34 - RNA, 21 nt, Artificial Sequence
  synthesized siRNA antisense sequence
  misc_feature (5)..(5): cm
  misc_feature (8)..(8): cm
  misc_feature (17)..(17): cm
  misc_feature (20)..(21): n=deoxythymidine
  misc_feature (20)..(21): phosphorothioate bond
guugcaucaaaugcuucagnn

SEQ ID NO: 35 - RNA, 21 nt, Artificial Sequence
  synthesized siRNA sense sequence
  misc_feature (1)..(2): um
  misc_feature (3)..(3): cm
  misc_feature (4)..(4): um
  misc_feature (6)..(6): cm
  misc_feature (9)..(9): cm
  misc_feature (10)..(10): um
  misc_feature (14)..(15): um
  misc_feature (16)..(16): cm
  misc_feature (19)..(19): um
  misc_feature (20)..(21): n=deoxythymidine
  misc_feature (20)..(21): phosphorothioate bond
uucugcaacugaauucgaunn

SEQ ID NO: 36 - RNA, 21 nt, Artificial Sequence
  synthesized siRNA antisense sequence
  misc_feature (9)..(9): cm
  misc_feature (15)..(15): cm
  misc_feature (20)..(21): n=deoxythymidine
  misc_feature (20)..(21): phosphorothioate bond
aucgaauucaguugcagaann

SEQ ID NO: 37 - RNA, 21 nt, Artificial Sequence
  synthesized siRNA sense sequence
  misc_feature (1)..(1): um
  misc_feature (10)..(10): cm
  misc_feature (11)..(11): um
  misc_feature (13)..(15): um
  misc_feature (17)..(17): cm
  misc_feature (20)..(21): n=deoxythymidine
  misc_feature (20)..(21): phosphorothioate bond
ugaaaggaacuguuuacaann

SEQ ID NO: 38 - RNA, 21 nt, Artificial Sequence
  synthesized siRNA antisense sequence
  misc_feature (4)..(4): cm
  misc_feature (8)..(8): cm
  misc_feature (18)..(18): cm
  misc_feature (20)..(21): n=deoxythymidine
  misc_feature (20)..(21): phosphorothioate bond
uuguaaacaguuccuuucann

SEQ ID NO: 39 - RNA, 21 nt, Artificial Sequence
  synthesized siRNA sense sequence
  misc_feature (2)..(2): cm
  misc_feature (3)..(3): um
  misc_feature (8)..(8): cm
  misc_feature (10)..(12): um
  misc_feature (15)..(15): um
  misc_feature (17)..(17): cm
  misc_feature (20)..(21): n=deoxythymidine
  misc_feature (20)..(21): phosphorothioate bond
acugaagcauuugaugcaann

SEQ ID NO: 40 - RNA, 21 nt, Artificial Sequence
  synthesized siRNA antisense sequence
  misc_feature (4)..(4): cm
  misc_feature (7)..(7): cm
  misc_feature (16)..(16): cm
  misc_feature (20)..(21): n=deoxythymidine
  misc_feature (20)..(21): phosphorothioate bond
uugcaucaaaugcuucagunn

SEQ ID NO: 41 - RNA, 21 nt, Artificial Sequence
  synthesized siRNA sense sequence
  misc_feature (1)..(1): cm
  misc_feature (3)..(3): um
  misc_feature (5)..(5): cm
  misc_feature (9)..(9): cm
  misc_feature (13)..(14): cm
  misc_feature (15)..(15): um
  misc_feature (17)..(19): um
  misc_feature (20)..(21): n=deoxythymidine
  misc_feature (20)..(21): phosphorothioate bond
cauacagacaaaccuguuunn

SEQ ID NO: 42 - RNA, 21 nt, Artificial Sequence
  synthesized siRNA antisense sequence
  misc_feature (4)..(4): cm
  misc_feature (16)..(16): um
  misc_feature (20)..(21): n=deoxythymidine
  misc_feature (20)..(21): phosphorothioate bond
aaacagguuugucuguaugnn

SEQ ID NO: 43 - RNA, 21 nt, Artificial Sequence
  synthesized siRNA sense sequence
  misc_feature (4)..(4): cm
  misc_feature (7)..(7): cm
  misc_feature (11)..(11): um
  misc_feature (13)..(14): cm
  misc_feature (15)..(17): um
  misc_feature (19)..(19): um
  misc_feature (20)..(21): n=deoxythymidine
  misc_feature (20)..(21): phosphorothioate bond
aaacaacaaguaccuuuaunn

SEQ ID NO: 44 - RNA, 21 nt, Artificial Sequence
  synthesized siRNA antisense sequence
  misc_feature (2)..(2): um
  misc_feature (8)..(8): um
  misc_feature (20)..(21): n=deoxythymidine
  misc_feature (20)..(21): phosphorothioate bond
auaaagguacuuguuguuunn

SEQ ID NO: 45 - RNA, 21 nt, Artificial Sequence
  synthesized siRNA sense sequence
  misc_feature (2)..(2): um
  misc_feature (4)..(4): cm
  misc_feature (8)..(8): cm
  misc_feature (12)..(13): cm
  misc_feature (14)..(14): um
  misc_feature (16)..(18): um
  misc_feature (20)..(21): n=deoxythymidine
  misc_feature (20)..(21): phosphorothioate bond
auacagacaaaccuguuuann

SEQ ID NO: 46 - RNA, 21 nt, Artificial Sequence
  synthesized siRNA antisense sequence
  misc_feature (1)..(1): um
  misc_feature (5)..(5): cm
  misc_feature (17)..(17): um
  misc_feature (20)..(21): n=deoxythymidine
  misc_feature (20)..(21): phosphorothioate bond
uaaacagguuugucuguaunn

SEQ ID NO: 47 - RNA, 21 nt, Artificial Sequence
  synthesized siRNA sense sequence
  misc_feature (3)..(3): um
  misc_feature (5)..(5): um
  misc_feature (7)..(7): um
  misc_feature (9)..(9): um
  misc_feature (11)..(12): um
  misc_feature (14)..(14): cm
  misc_feature (15)..(15): um
  misc_feature (18)..(18): um
  misc_feature (20)..(21): n=deoxythymidine
  misc_feature (20)..(21): phosphorothioate bond
gguauauguguugcugauann

SEQ ID NO: 48 - RNA, 21 nt, Artificial Sequence
  synthesized siRNA antisense sequence
  misc_feature (1)..(1): um
  misc_feature (4)..(4): cm
  misc_feature (7)..(7): cm
  misc_feature (10)..(10): cm
  misc_feature (12)..(12): cm
  misc_feature (14)..(14): um
  misc_feature (16)..(16): um
  misc_feature (20)..(21): n=deoxythymidine
  misc_feature (20)..(21): phosphorothioate bond
uaucagcaacacauauaccnn

SEQ ID NO: 49 - RNA, 21 nt, Artificial Sequence
  synthesized siRNA sense sequence
  misc_feature (1)..(1): um
  misc_feature (2)..(2): cm
  misc_feature (9)..(9): um
  misc_feature (10)..(10): cm
  misc_feature (11)..(11): um
  misc_feature (13)..(13): um
  misc_feature (20)..(21): n=deoxythymidine
  misc_feature (20)..(21): phosphorothioate bond
ucagaaagucugugaaggann

SEQ ID NO: 50 - RNA, 21 nt, Artificial Sequence
  synthesized siRNA antisense sequence
  misc_feature (6)..(6): cm
  misc_feature (8)..(8): cm
  misc_feature (20)..(21): n=deoxythymidine
  misc_feature (20)..(21): phosphorothioate bond
uccuucacagacuuucugann

SEQ ID NO: 51 - RNA, 21 nt, Artificial Sequence
  synthesized siRNA sense sequence
  misc_feature (1)..(1): um
  misc_feature (2)..(2): cm
  misc_feature (3)..(3): um
  misc_feature (4)..(5): cm
  misc_feature (9)..(10): cm
  misc_feature (14)..(14): cm
  misc_feature (15)..(15): um
  misc_feature (17)..(17): um
  misc_feature (19)..(19): um
  misc_feature (20)..(21): n=deoxythymidine
  misc_feature (20)..(21): phosphorothioate bond
ucuccaggccaaacugugunn

SEQ ID NO: 52 - RNA, 21 nt, Artificial Sequence
  synthesized siRNA antisense sequence
  misc_feature (2)..(2): cm
  misc_feature (4)..(4): cm
  misc_feature (20)..(21): n=deoxythymidine
  misc_feature (20)..(21): phosphorothioate bond
acacaguuuggccuggagann

SEQ ID NO: 53 - RNA, 21 nt, Artificial Sequence
  synthesized siRNA sense sequence
  misc_feature (2)..(2): cm
  misc_feature (5)..(5): cm
  misc_feature (9)..(9): um
  misc_feature (11)..(12): cm
  misc_feature (13)..(15): um
  misc_feature (17)..(17): um
  misc_feature (19)..(19): um
  misc_feature (20)..(21): n=deoxythymidine
  misc_feature (20)..(21): phosphorothioate bond
acaacaaguaccuuuauaunn

SEQ ID NO: 54 - RNA, 21 nt, Artificial Sequence
  synthesized siRNA antisense sequence
  misc_feature (2)..(2): um
  misc_feature (4)..(4): um
  misc_feature (10)..(10): um
  misc_feature (20)..(21): n=deoxythymidine
  misc_feature (20)..(21): phosphorothioate bond
auauaaagguacuuguugunn

SEQ ID NO: 55 - RNA, 21 nt, Artificial Sequence
  synthesized siRNA sense sequence
  misc_feature (1)..(1): cm
  misc_feature (4)..(4): cm
  misc_feature (8)..(8): um
  misc_feature (10)..(11): cm
  misc_feature (12)..(14): um
  misc_feature (16)..(16): um
  misc_feature (18)..(19): um
  misc_feature (20)..(21): n=deoxythymidine
  misc_feature (20)..(21): phosphorothioate bond
caacaaguaccuuuauauunn

SEQ ID NO: 56 - RNA, 21 nt, Artificial Sequence
  synthesized siRNA antisense sequence
  misc_feature (3)..(3): um
  misc_feature (5)..(5): um
  misc_feature (11)..(11): um
  misc_feature (20)..(21): n=deoxythymidine
  misc_feature (20)..(21): phosphorothioate bond
aauauaaagguacuuguugnn

SEQ ID NO: 57 - RNA, 21 nt, Artificial Sequence
  synthesized siRNA sense sequence
  misc_feature (2)..(3): um
  misc_feature (4)..(4): cm
  misc_feature (5)..(5): um
  misc_feature (6)..(7): cm
  misc_feature (11)..(12): cm
  misc_feature (16)..(16): cm
  misc_feature (17)..(17): um
  misc_feature (19)..(19): um
  misc_feature (20)..(21): n=deoxythymidine
  misc_feature (20)..(21): phosphorothioate bond
auucuccaggccaaacugunn

SEQ ID NO: 58 - RNA, 21 nt, Artificial Sequence
  synthesized siRNA antisense sequence
  misc_feature (2)..(2): cm
  misc_feature (20)..(21): n=deoxythymidine
  misc_feature (20)..(21): phosphorothioate bond
acaguuuggccuggagaaunn

SEQ ID NO: 59 - RNA, 21 nt, Artificial Sequence
  synthesized siRNA sense sequence
  misc_feature (2)..(2): um
  misc_feature (5)..(5): cm
  misc_feature (8)..(9): cm
  misc_feature (12)..(12): cm
  misc_feature (13)..(13): um
  misc_feature (14)..(15): cm
  misc_feature (19)..(19): um
  misc_feature (20)..(21): n=deoxythymidine
  misc_feature (20)..(21): phosphorothioate bond
guggcaaccagcuccaggunn

SEQ ID NO: 60 - RNA, 21 nt, Artificial Sequence
  synthesized siRNA antisense sequence
  misc_feature (17)..(17): cm
  misc_feature (20)..(21): n=deoxythymidine
  misc_feature (20)..(21): phosphorothioate bond
accuggagcugguugccacnn

SEQ ID NO: 61 - RNA, 21 nt, Artificial Sequence
  synthesized siRNA sense sequence
  misc_feature (7)..(7): cm
  misc_feature (9)..(9): um
  misc_feature (10)..(10): cm
  misc_feature (11)..(11): um
  misc_feature (14)..(14): cm
  misc_feature (15)..(16): um
  misc_feature (20)..(21): n=deoxythymidine
  misc_feature (20)..(21): phosphorothioate bond
aagagacaucugacuuggann

SEQ ID NO: 62 - RNA, 21 nt, Artificial Sequence
  synthesized siRNA antisense sequence
  misc_feature (3)..(3): cm
  misc_feature (8)..(8): cm
  misc_feature (20)..(21): n=deoxythymidine
  misc_feature (20)..(21): phosphorothioate bond
uccaagucagaugucucuunn

SEQ ID NO: 63 - RNA, 21 nt, Artificial Sequence
  synthesized siRNA sense sequence
  misc_feature (2)..(3): um
  misc_feature (4)..(4): cm
  misc_feature (5)..(5): um
  misc_feature (7)..(7): cm
  misc_feature (10)..(10): cm
  misc_feature (11)..(11): um
  misc_feature (15)..(16): um
  misc_feature (17)..(17): cm
  misc_feature (20)..(21): n=deoxythymidine
  misc_feature (20)..(21): phosphorothioate bond
auucugcaacugaauucgann

SEQ ID NO: 64 - RNA, 21 nt, Artificial Sequence
  synthesized siRNA antisense sequence
  misc_feature (8)..(8): cm
  misc_feature (14)..(14): cm
  misc_feature (20)..(21): n=deoxythymidine
  misc_feature (20)..(21): phosphorothioate bond
ucgaauucaguugcagaaunn

SEQ ID NO: 65 - RNA, 21 nt, Artificial Sequence
  synthesized siRNA sense sequence
  misc_feature (1)..(2): um
  misc_feature (3)..(4): cm
  misc_feature (5)..(5): um
  misc_feature (6)..(6): cm
  misc_feature (7)..(7): um
  misc_feature (13)..(14): um
  misc_feature (17)..(18): cm
  misc_feature (19)..(19): um
  misc_feature (20)..(21): n=deoxythymidine
  misc_feature (20)..(21): phosphorothioate bond
uuccucuggaaauuggccunn

SEQ ID NO: 66 - RNA, 21 nt, Artificial Sequence
  synthesized siRNA antisense sequence
  misc_feature (5)..(5): cm
  misc_feature (12)..(12): cm
  misc_feature (20)..(21): n=deoxythymidine
  misc_feature (20)..(21): phosphorothioate bond
aggccaauuuccagaggaann

SEQ ID NO: 67 - RNA, 21 nt, Artificial Sequence
  synthesized siRNA sense sequence
  misc_feature (3)..(3): cm
  misc_feature (6)..(6): cm
  misc_feature (10)..(10): um
  misc_feature (12)..(13): cm
  misc_feature (14)..(16): um
  misc_feature (18)..(18): um
  misc_feature (20)..(21): n=deoxythymidine
  misc_feature (20)..(21): phosphorothioate bond
aacaacaaguaccuuuauann

SEQ ID NO: 68 - RNA, 21 nt, Artificial Sequence
  synthesized siRNA antisense sequence
  misc_feature (1)..(1): um
  misc_feature (3)..(3): um
  misc_feature (9)..(9): um
  misc_feature (20)..(21): n=deoxythymidine
  misc_feature (20)..(21): phosphorothioate bond
uauaaagguacuuguuguunn

SEQ ID NO: 69 - RNA, 21 nt, Artificial Sequence
  synthesized siRNA sense sequence
  misc_feature (3)..(3): um
  misc_feature (5)..(5): um
  misc_feature (7)..(7): um
  misc_feature (8)..(9): cm
  misc_feature (10)..(10): um
  misc_feature (11)..(11): cm
  misc_feature (12)..(12): um
  misc_feature (13)..(13): cm
  misc_feature (14)..(14): um
  misc_feature (15)..(17): cm
  misc_feature (18)..(18): um
  misc_feature (20)..(21): n=deoxythymidine
  misc_feature (20)..(21): phosphorothioate bond
aauauguccucucucccuann

SEQ ID NO: 70 - RNA, 21 nt, Artificial Sequence
  synthesized siRNA antisense sequence
  misc_feature (1)..(1): um
  misc_feature (14)..(14): cm
  misc_feature (16)..(16): um
  misc_feature (20)..(21): n=deoxythymidine
  misc_feature (20)..(21): phosphorothioate bond
uagggagagaggacauauunn

SEQ ID NO: 71 - RNA, 21 nt, Artificial Sequence
  synthesized siRNA sense sequence
  misc_feature (2)..(2): cm
  misc_feature (3)..(3): um
  misc_feature (4)..(4): cm
  misc_feature (6)..(6): cm
  misc_feature (7)..(7): um
  misc_feature (9)..(9): um
  misc_feature (12)..(13): um
  misc_feature (15)..(15): cm
  misc_feature (16)..(17): um
  misc_feature (20)..(21): n=deoxythymidine
  misc_feature (20)..(21): phosphorothioate bond
acucacuauaauuacuugann

SEQ ID NO: 72 - RNA, 21 nt, Artificial Sequence
  synthesized siRNA antisense sequence
  misc_feature (2)..(2): cm
  misc_feature (6)..(6): um
  misc_feature (10)..(10): um
  misc_feature (12)..(12): um
  misc_feature (20)..(21): n=deoxythymidine
  misc_feature (20)..(21): phosphorothioate bond
ucaaguaauuauagugagunn

SEQ ID NO: 73 - RNA, 21 nt, Artificial Sequence
  synthesized siRNA sense sequence
  misc_feature (2)..(2): um
  misc_feature (5)..(5): cm
  misc_feature (6)..(6): um
  misc_feature (7)..(7): cm
  misc_feature (9)..(9): cm
  misc_feature (10)..(10): um
  misc_feature (12)..(12): um
  misc_feature (15)..(16): um
  misc_feature (18)..(18): cm
  misc_feature (19)..(19): um
  misc_feature (20)..(21): n=deoxythymidine
  misc_feature (20)..(21): phosphorothioate bond
auaacucacuauaauuacunn

SEQ ID NO: 74 - RNA, 21 nt, Artificial Sequence
  synthesized siRNA antisense sequence
  misc_feature (3)..(3): um
  misc_feature (7)..(7): um
  misc_feature (9)..(9): um
  misc_feature (17)..(17): um
  misc_feature (20)..(21): n=deoxythymidine
  misc_feature (20)..(21): phosphorothioate bond
aguaauuauagugaguuaunn

SEQ ID NO: 75 - RNA, 21 nt, Artificial Sequence
  synthesized siRNA sense sequence
  misc_feature (4)..(4): um
  misc_feature (6)..(6): um
  misc_feature (8)..(8): um
  misc_feature (9)..(10): cm
  misc_feature (11)..(11): um
  misc_feature (12)..(12): cm
  misc_feature (13)..(13): um
  misc_feature (14)..(14): cm
  misc_feature (15)..(15): um
  misc_feature (16)..(18): cm
  misc_feature (19)..(19): um
  misc_feature (20)..(21): n=deoxythymidine
  misc_feature (20)..(21): phosphorothioate bond
aaauauguccucucucccunn

SEQ ID NO: 76 - RNA, 21 nt, Artificial Sequence
  synthesized siRNA antisense sequence
  misc_feature (13)..(13): cm
  misc_feature (15)..(15): um
  misc_feature (20)..(21): n=deoxythymidine
  misc_feature (20)..(21): phosphorothioate bond
agggagagaggacauauuunn

SEQ ID NO: 77 - RNA, 21 nt, Artificial Sequence
  synthesized siRNA sense sequence
  misc_feature (5)..(5): um
  misc_feature (7)..(11): um
  misc_feature (13)..(13): um
  misc_feature (16)..(16): um
  misc_feature (20)..(21): n=deoxythymidine
  misc_feature (20)..(21): phosphorothioate bond
aagauauuuuuauaauaaann

SEQ ID NO: 78 - RNA, 21 nt, Artificial Sequence
  synthesized siRNA antisense sequence
  misc_feature (3)..(3): um
  misc_feature (6)..(6): um
  misc_feature (8)..(8): um
  misc_feature (14)..(14): um
  misc_feature (20)..(21): n=deoxythymidine
  misc_feature (20)..(21): phosphorothioate bond
uuuauuauaaaaauaucuunn

SEQ ID NO: 79 - RNA, 21 nt, Artificial Sequence
  synthesized siRNA sense sequence
  misc_feature (5)..(5): um
  misc_feature (8)..(8): cm
  misc_feature (9)..(9): um
  misc_feature (10)..(10): cm
  misc_feature (12)..(12): cm
  misc_feature (13)..(13): um
  misc_feature (15)..(15): um
  misc_feature (18)..(19): um
  misc_feature (20)..(21): n=deoxythymidine
  misc_feature (20)..(21): phosphorothioate bond
aaaauaacucacuauaauunn

SEQ ID NO: 80 - RNA, 21 nt, Artificial Sequence
  synthesized siRNA antisense sequence
  misc_feature (4)..(4): um
  misc_feature (6)..(6): um
  misc_feature (14)..(14): um
  misc_feature (20)..(21): n=deoxythymidine
  misc_feature (20)..(21): phosphorothioate bond
aauuauagugaguuauuuunn

SEQ ID NO: 81 - RNA, 21 nt, Artificial Sequence
  synthesized siRNA sense sequence
  misc_feature (4)..(4): um
  misc_feature (7)..(7): cm
  misc_feature (8)..(8): um
  misc_feature (9)..(9): cm
  misc_feature (11)..(11): cm
  misc_feature (12)..(12): um
  misc_feature (14)..(14): um
  misc_feature (17)..(18): um
  misc_feature (20)..(21): n=deoxythymidine
  misc_feature (20)..(21): phosphorothioate bond
aaauaacucacuauaauuann

SEQ ID NO: 82 - RNA, 21 nt, Artificial Sequence
  synthesized siRNA antisense sequence
  misc_feature (1)..(1): um
  misc_feature (5)..(5): um
  misc_feature (7)..(7): um
  misc_feature (15)..(15): um
  misc_feature (20)..(21): n=deoxythymidine
  misc_feature (20)..(21): phosphorothioate bond
uaauuauagugaguuauuunn

SEQ ID NO: 83 - RNA, 21 nt, Artificial Sequence
  synthesized siRNA sense sequence
  misc_feature (2)..(2): um
  misc_feature (4)..(5): um
  misc_feature (10)..(10): um
  misc_feature (12)..(12): um
  misc_feature (13)..(13): cm
  misc_feature (14)..(14): um
  misc_feature (16)..(16): cm
  misc_feature (17)..(17): um
  misc_feature (19)..(19): um
  misc_feature (20)..(21): n=deoxythymidine
  misc_feature (20)..(21): phosphorothioate bond
guguuaaaaugucugcugunn

SEQ ID NO: 84 - RNA, 21 nt, Artificial Sequence
  synthesized siRNA antisense sequence
  misc_feature (2)..(2): cm
  misc_feature (5)..(5): cm
  misc_feature (9)..(9): cm
  misc_feature (14)..(14): um
  misc_feature (17)..(17): cm
  misc_feature (20)..(21): n=deoxythymidine
  misc_feature (20)..(21): phosphorothioate bond
acagcagacauuuuaacacnn

SEQ ID NO: 85 - RNA, 21 nt, Artificial Sequence
  synthesized siRNA sense sequence
  misc_feature (5)..(5): um
  misc_feature (7)..(11): um
  misc_feature (13)..(13): um
  misc_feature (14)..(14): cm
  misc_feature (18)..(18): um
  misc_feature (20)..(21): n=deoxythymidine
  misc_feature (20)..(21): phosphorothioate bond
aaaauguuuuugucaaguann

SEQ ID NO: 86 - RNA, 21 nt, Artificial Sequence
  synthesized siRNA antisense sequence
  misc_feature (1)..(1): um
  misc_feature (8)..(8): cm
  misc_feature (14)..(14): cm
  misc_feature (20)..(21): n=deoxythymidine
  misc_feature (20)..(21): phosphorothioate bond
uacuugacaaaaacauuuunn

SEQ ID NO: 87 - RNA, 21 nt, Artificial Sequence
  synthesized siRNA sense sequence
  misc_feature (1)..(1): cm
  misc_feature (2)..(3): um
  misc_feature (5)..(5): cm
  misc_feature (7)..(7): cm
  misc_feature (8)..(8): um
  misc_feature (12)..(12): um
  misc_feature (14)..(14): cm
  misc_feature (15)..(16): um
  misc_feature (17)..(17): cm
  misc_feature (20)..(21): n=deoxythymidine
  misc_feature (20)..(21): phosphorothioate bond
cuuacgcugaguacuucgann

SEQ ID NO: 88 - RNA, 21 nt, Artificial Sequence
  synthesized siRNA antisense sequence
  misc_feature (7)..(7): um
  misc_feature (11)..(11): cm
  misc_feature (16)..(16): um
  misc_feature (20)..(21): n=deoxythymidine
  misc_feature (20)..(21): phosphorothioate bond
ucgaaguacucagcguaagnn

SEQ ID NO: 89 - RNA, 21 nt, Artificial Sequence
  synthesized siRNA sense sequence
  misc_feature (4)..(4): cm
  misc_feature (10)..(10): um
  misc_feature (12)..(13): um
  misc_feature (14)..(14): cm
  misc_feature (20)..(21): n=deoxythymidine
  misc_feature (20)..(21): phosphorothioate bond
aggcaaagguguucaaagann

SEQ ID NO: 90 - RNA, 21 nt, Artificial Sequence
  synthesized siRNA antisense sequence
  misc_feature (9)..(9): cm
  misc_feature (20)..(21): n=deoxythymidine
  misc_feature (20)..(21): phosphorothioate bond
ucuuugaacaccuuugccunn

SEQ ID NO: 91 - RNA, 19 nt, Artificial Sequence
  synthesized siRNA sense sequence
  misc_feature (4)..(4): cm
  misc_feature (10)..(10): um
  misc_feature (12)..(13): um
  misc_feature (14)..(14): cm
aggcaaagguguucaaaga

SEQ ID NO: 92 - RNA, 19 nt, Artificial Sequence
  synthesized siRNA antisense sequence
  misc_feature (9)..(9): cm
ucuuugaacaccuuugccu

SEQ ID NO: 93 - RNA, 21 nt, Artificial Sequence
  synthesized siRNA sense sequence
  misc_feature (1)..(2): phosphorothioate bond
  misc_feature (4)..(4): cm
  misc_feature (10)..(10): um
  misc_feature (10)..(21): um
  misc_feature (12)..(13): um
  misc_feature (14)..(14): cm
aggcaaagguguucaaagauu

SEQ ID NO: 94 - RNA, 21 nt, Artificial Sequence
  synthesized siRNA antisense sequence
  misc_feature (1)..(2): phosphorothioate bond
  misc_feature (9)..(9): cm
  misc_feature (20)..(21): um
ucuuugaacaccuuugccuuu

SEQ ID NO: 95 - RNA, 21 nt, Artificial Sequence
  synthesized siRNA sense sequence
  misc_feature (1)..(2): phosphorothioate bond
  misc_feature (2)..(3): phosphorothioate bond
  misc_feature (4)..(4): cm
  misc_feature (10)..(10): um
  misc_feature (12)..(13): um
  misc_feature (14)..(14): cm
  misc_feature (20)..(21): um
aggcaaagguguucaaagauu

SEQ ID NO: 96 - RNA, 21 nt, Artificial Sequence
  synthesized siRNA antisense sequence
  misc_feature (1)..(3): phosphorothioate bond
  misc_feature (9)..(9): cm
  misc_feature (20)..(21): um
ucuuugaacaccuuugccuuu

SEQ ID NO: 97 - RNA, 21 nt, Artificial Sequence
  synthesized siRNA sense sequence
  misc_feature (1)..(2): phosphorothioate bond
  misc_feature (4)..(4): cm
  misc_feature (10)..(10): um
  misc_feature (12)..(13): um
  misc_feature (14)..(14): cm
  misc_feature (19)..(20): phosphorothioate bond
  misc_feature (20)..(21): phosphorothioate bond
  misc_feature (20)..(21): um
aggcaaagguguucaaagauu

SEQ ID NO: 98 - RNA, 21 nt, Artificial Sequence
  synthesized siRNA antisense sequence
  misc_feature (1)..(2): phosphorothioate bond
  misc_feature (9)..(9): cm
  misc_feature (19)..(21): phosphorothioate bond
  misc_feature (20)..(21): um
ucuuugaacaccuuugccuuu

SEQ ID NO: 99 - RNA, 19 nt, Artificial Sequence
  synthesized siRNA sense sequence
  misc_feature (4)..(4): cm
  misc_feature (10)..(10): um
  misc_feature (12)..(13): um
  misc_feature (14)..(14): cm
aggcaaagguguucaaaga

SEQ ID NO: 100 - RNA, 21 nt, Artificial Sequence
  synthesized siRNA antisense sequence
  misc_feature (9)..(9): cm
  misc_feature (20)..(21): um
ucuuugaacaccuuugccuuu

SEQ ID NO: 101 - RNA, 21 nt, Artificial Sequence
  synthesized siRNA sense sequence
  misc_feature (2)..(2): um
  misc_feature (6)..(6): cm
  misc_feature (12)..(12): um
  misc_feature (14)..(15): um
  misc_feature (16)..(16): cm
auaggcaaagguguucaaaga

SEQ ID NO: 102 - RNA, 21 nt, Artificial Sequence
  synthesized siRNA antisense sequence
  misc_feature (9)..(9): cm
  misc_feature (20)..(21): um
ucuuugaacaccuuugccuuu

SEQ ID NO: 103 - skipped

SEQ ID NO: 104 - RNA, 21 nt, Artificial Sequence
  synthesized siRNA antisense sequence
  misc_feature (9)..(9): cm
  misc_feature (20)..(21): um
ucuuugaacaccuuugccuuu

SEQ ID NO: 105 - skipped

SEQ ID NO: 106 - RNA, 21 nt, Artificial Sequence
  synthesized siRNA antisense sequence
  misc_feature (8)..(8): cm
  misc_feature (20)..(21): n=deoxythymidine
  misc_feature (20)..(21): phosphorothioate bond
cuuugaacaccuuugccuunn

SEQ ID NO: 107 - RNA, 19 nt, Artificial Sequence
  synthesized siRNA sense sequence
  misc_feature (5)..(5): cm
  misc_feature (11)..(11): um
  misc_feature (13)..(14): um
  misc_feature (15)..(15): cm
aaggcaaagguguucaaag

SEQ ID NO: 108 - RNA, 19 nt, Artificial Sequence
  synthesized siRNA antisense sequence
  misc_feature (8)..(8): cm
cuuugaacaccuuugccuu

SEQ ID NO: 109 - RNA, 21 nt, Artificial Sequence
  synthesized siRNA sense sequence
  misc_feature (9)..(9): cm
  misc_feature (10)..(10): um
  misc_feature (12)..(14): um
  misc_feature (16)..(16): cm
  misc_feature (19)..(19): cm
  misc_feature (20)..(21): n=deoxythymidine
  misc_feature (20)..(21): phosphorothioate bond
gaaaggaacuguuuacaacnn

SEQ ID NO: 110 - RNA, 21 nt, Artificial Sequence
  synthesized siRNA antisense sequence
  misc_feature (5)..(5): um
  misc_feature (9)..(9): cm
  misc_feature (20)..(21): n=deoxythymidine
  misc_feature (20)..(21): phosphorothioate bond
guuguaaacaguuccuuucnn

SEQ ID NO: 111 - RNA, 19 nt, Artificial Sequence
  synthesized siRNA sense sequence
  misc_feature (9)..(9): cm
  misc_feature (10)..(10): um
  misc_feature (13)..(15): um
  misc_feature (17)..(17): cm
  misc_feature (19)..(19): cm
gaaaggaacuguuuacaac

SEQ ID NO: 112 - RNA, 19 nt, Artificial Sequence
  synthesized siRNA antisense sequence
  misc_feature (5)..(5): um
  misc_feature (9)..(9): cm
guuguaaacaguuccuuuc

SEQ ID NO: 113 - RNA, 21 nt, Artificial Sequence
  synthesized siRNA sense sequence
  misc_feature (1)..(1): um
  misc_feature (4)..(4): um
  misc_feature (6)..(6): um
  misc_feature (8)..(8): um
  misc_feature (10)..(10): um
  misc_feature (12)..(13): um
  misc_feature (15)..(15): cm
  misc_feature (16)..(16): um
  misc_feature (19)..(19): um
  misc_feature (20)..(21): n=deoxythymidine
  misc_feature (20)..(21): phosphorothioate bond
ugguauauguguugcugaunn

SEQ ID NO: 114 - RNA, 21 nt, Artificial Sequence
  synthesized siRNA antisense sequence
  misc_feature (3)..(3): cm
  misc_feature (6)..(6): cm
  misc_feature (9)..(9): cm
  misc_feature (11)..(11): cm
  misc_feature (13)..(13): um
  misc_feature (15)..(15): um
  misc_feature (18)..(18): cm
  misc_feature (20)..(21): n=deoxythymidine
  misc_feature (20)..(21): phosphorothioate bond
aucagcaacacauauaccann

SEQ ID NO: 115 - RNA, 19 nt, Artificial Sequence
  synthesized siRNA sense sequence
  misc_feature (1)..(1): um
  misc_feature (4)..(4): um
  misc_feature (6)..(6): um
  misc_feature (8)..(8): um
  misc_feature (10)..(10): um
  misc_feature (12)..(13): um
  misc_feature (15)..(15): cm
  misc_feature (16)..(16): um
  misc_feature (19)..(19): um
ugguauauguguugcugau

SEQ ID NO: 116 - RNA, 19 nt, Artificial Sequence
  synthesized siRNA antisense sequence
  misc_feature (3)..(3): cm
  misc_feature (6)..(6): cm
  misc_feature (9)..(9): cm
  misc_feature (11)..(11): cm
  misc_feature (13)..(13): um
  misc_feature (15)..(15): um
  misc_feature (18)..(18): cm
aucagcaacacauauacca

SEQ ID NO: 117 - RNA, 21 nt, Artificial Sequence
  synthesized siRNA sense sequence
  misc_feature (1)..(1): um
  misc_feature (1)..(2): phosphorothioate bond
  misc_feature (4)..(4): um
  misc_feature (6)..(6): um
  misc_feature (8)..(8): um
  misc_feature (10)..(10): um
  misc_feature (12)..(13): um
  misc_feature (15)..(15): cm
  misc_feature (16)..(16): um
  misc_feature (19)..(21): um
ugguauauguguugcugauuu

SEQ ID NO: 118 - RNA, 21 nt, Artificial Sequence
  synthesized siRNA antisense sequence
  misc_feature (1)..(2): phosphorothioate bond
  misc_feature (3)..(3): cm
  misc_feature (6)..(6): cm
  misc_feature (9)..(9): cm
  misc_feature (11)..(11): cm
  misc_feature (13)..(13): um
  misc_feature (15)..(15): um
  misc_feature (18)..(18): cm
  misc_feature (20)..(21): um
aucagcaacacauauaccauu

SEQ ID NO: 119 - RNA, 21 nt, Artificial Sequence
  synthesized siRNA sense sequence
  misc_feature (1)..(3): phosphorothioate bond
  misc_feature (1)..(1): um
  misc_feature (4)..(4): um
  misc_feature (6)..(6): um
  misc_feature (8)..(8): um
  misc_feature (10)..(10): um
  misc_feature (12)..(13): um
  misc_feature (15)..(15): cm
  misc_feature (16)..(16): um
  misc_feature (19)..(21): um
ugguauauguguugcugauuu

SEQ ID NO: 120 - RNA, 21 nt, Artificial Sequence
  synthesized siRNA antisense sequence
  misc_feature (1)..(3): phosphorothioate bond
  misc_feature (3)..(3): cm
  misc_feature (6)..(6): cm
  misc_feature (9)..(9): cm
  misc_feature (11)..(11): cm
  misc_feature (13)..(13): um
  misc_feature (15)..(15): um
  misc_feature (18)..(18): cm
  misc_feature (20)..(21): um
aucagcaacacauauaccauu

SEQ ID NO: 121 - RNA, 21 nt, Artificial Sequence
  synthesized siRNA sense sequence
  misc_feature (1)..(1): um
  misc_feature (1)..(2): phosphorothioate bond
  misc_feature (4)..(4): um
  misc_feature (6)..(6): um
  misc_feature (8)..(8): um
  misc_feature (10)..(10): um
  misc_feature (12)..(13): um
  misc_feature (15)..(15): cm
  misc_feature (16)..(16): um
  misc_feature (19)..(21): um
  misc_feature (19)..(21): phosphorothioate bond
ugguauauguguugcugauuu

SEQ ID NO: 122 - RNA, 21 nt, Artificial Sequence
  synthesized siRNA antisense sequence
  misc_feature (1)..(2): phosphorothioate bond
  misc_feature (3)..(3): cm
  misc_feature (6)..(6): cm
  misc_feature (9)..(9): cm
  misc_feature (11)..(11): cm
  misc_feature (13)..(13): um
  misc_feature (15)..(15): um
  misc_feature (18)..(18): cm
  misc_feature (19)..(21): phosphorothioate bond
  misc_feature (20)..(21): um
aucagcaacacauauaccauu

SEQ ID NO: 123 - RNA, 19 nt, Artificial Sequence
  synthesized siRNA sense sequence
  misc_feature (1)..(1): um
  misc_feature (4)..(4): um
  misc_feature (6)..(6): um
  misc_feature (8)..(8): um
  misc_feature (10)..(10): um
  misc_feature (12)..(13): um
  misc_feature (15)..(15): cm
  misc_feature (16)..(16): um
  misc_feature (19)..(19): um
ugguauauguguugcugau

SEQ ID NO: 124 - RNA, 21 nt, Artificial Sequence
  synthesized siRNA antisense sequence
  misc_feature (3)..(3): cm
  misc_feature (6)..(6): cm
  misc_feature (9)..(9): cm
  misc_feature (11)..(11): cm
  misc_feature (13)..(13): um
  misc_feature (15)..(15): um
  misc_feature (18)..(18): cm
  misc_feature (20)..(21): um
aucagcaacacauauaccauu

SEQ ID NO: 125 - RNA, 21 nt, Artificial Sequence
  synthesized siRNA sense sequence
  misc_feature (2)..(3): um
  misc_feature (6)..(6): um
  misc_feature (8)..(8): um
  misc_feature (10)..(10): um
  misc_feature (12)..(12): um
  misc_feature (14)..(15): um
  misc_feature (17)..(17): cm
  misc_feature (18)..(18): um
  misc_feature (21)..(21): um
auugguauauguguugcugau

SEQ ID NO: 126 - RNA, 21 nt, Artificial Sequence
  synthesized siRNA antisense sequence
  misc_feature (3)..(3): cm
  misc_feature (6)..(6): cm
  misc_feature (9)..(9): cm
  misc_feature (11)..(11): cm
  misc_feature (13)..(13): um
  misc_feature (15)..(15): um
  misc_feature (18)..(18): cm
  misc_feature (20)..(21): um
aucagcaacacauauaccauu

SEQ ID NO: 127 - RNA, 22 nt, Artificial Sequence
  synthesized siRNA sense sequence
  misc_feature (1)..(1): um
  misc_feature (3)..(4): um
  misc_feature (7)..(7): um
  misc_feature (9)..(9): um
  misc_feature (11)..(11): um
  misc_feature (13)..(13): um
  misc_feature (15)..(16): um
  misc_feature (18)..(18): cm
  misc_feature (19)..(19): um
  misc_feature (22)..(22): um
uauugguauauguguugcugau

SEQ ID NO: 128 - RNA, 21 nt, Artificial Sequence
  synthesized siRNA antisense sequence
  misc_feature (3)..(3): cm
  misc_feature (6)..(6): cm
  misc_feature (9)..(9): cm
  misc_feature (11)..(11): cm
  misc_feature (13)..(13): um
  misc_feature (15)..(15): um
  misc_feature (18)..(18): cm
  misc_feature (20)..(21): um
aucagcaacacauauaccauu

SEQ ID NO: 129 - RNA, 23 nt, Artificial Sequence
  synthesized siRNA sense sequence
  misc_feature (1)..(1): um
  misc_feature (3)..(4): um
  misc_feature (7)..(7): um
  misc_feature (9)..(9): um
  misc_feature (11)..(11): um
  misc_feature (13)..(13): um
  misc_feature (15)..(16): um
  misc_feature (18)..(18): cm
  misc_feature (19)..(19): um
  misc_feature (22)..(22): um
  misc_feature (23)..(23): n=Inverted deoxythymidine
uauugguauauguguugcugaun

SEQ ID NO: 130 - RNA, 21 nt, Artificial Sequence
  synthesized siRNA antisense sequence
  misc_feature (3)..(3): cm
  misc_feature (6)..(6): cm
  misc_feature (9)..(9): cm
  misc_feature (11)..(11): cm
  misc_feature (13)..(13): um
  misc_feature (15)..(15): um
  misc_feature (18)..(18): cm
  misc_feature (20)..(21): um
aucagcaacacauauaccauu

SEQ ID NO: 131 - RNA, 21 nt, Artificial Sequence
  synthesized siRNA sense sequence
  misc_feature (1)..(1): um
  misc_feature (4)..(4): um
  misc_feature (6)..(6): um
  misc_feature (8)..(8): um
  misc_feature (10)..(10): um
  misc_feature (12)..(13): um
  misc_feature (16)..(16): um
  misc_feature (19)..(21): um
ugguauauguguugcugauuu

SEQ ID NO: 132 - RNA, 21 nt, Artificial Sequence
  synthesized siRNA antisense sequence
  misc_feature (3)..(3): cm
  misc_feature (6)..(6): cm
  misc_feature (9)..(9): cm
  misc_feature (11)..(11): cm
  misc_feature (13)..(13): um
  misc_feature (15)..(15): um
  misc_feature (18)..(18): cm
  misc_feature (20)..(21): um
aucagcaacacauauaccauu

SEQ ID NO: 133 - RNA, 21 nt, Artificial Sequence
  synthesized siRNA sense sequence
  misc_feature (1)..(1): um
  misc_feature (4)..(4): um
  misc_feature (6)..(6): um
  misc_feature (8)..(8): um
  misc_feature (10)..(10): um
  misc_feature (12)..(13): um
  misc_feature (15)..(15): cm
  misc_feature (19)..(21): um
ugguauauguguugcugauuu

SEQ ID NO: 134 - RNA, 21 nt, Artificial Sequence
  synthesized siRNA antisense sequence
  misc_feature (3)..(3): cm
  misc_feature (6)..(6): cm
  misc_feature (9)..(9): cm
  misc_feature (11)..(11): cm
  misc_feature (13)..(13): um
  misc_feature (15)..(15): um
  misc_feature (18)..(18): cm
  misc_feature (20)..(21): um
aucagcaacacauauaccauu

SEQ ID NO: 135 - RNA, 20 nt, Artificial Sequence
  synthesized siRNA sense sequence
  misc_feature (2)..(3): um
  misc_feature (6)..(6): um
  misc_feature (8)..(8): um
  misc_feature (10)..(10): um
  misc_feature (12)..(12): um
  misc_feature (14)..(15): um
  misc_feature (17)..(17): cm
  misc_feature (18)..(18): um
auugguauauguguugcuga

SEQ ID NO: 136 - RNA, 20 nt, Artificial Sequence
  synthesized siRNA antisense sequence
  misc_feature (2)..(2): cm
  misc_feature (5)..(5): cm
  misc_feature (8)..(8): cm
  misc_feature (10)..(10): cm
  misc_feature (12)..(12): um
  misc_feature (14)..(14): um
  misc_feature (17)..(17): cm
  misc_feature (19)..(20): um
ucagcaacacauauaccauu

SEQ ID NO: 137 - RNA, 20 nt, Artificial Sequence
  synthesized siRNA sense sequence
  misc_feature (2)..(2): um
  misc_feature (5)..(5): um
  misc_feature (7)..(7): um
  misc_feature (9)..(9): um
  misc_feature (11)..(11): um
  misc_feature (13)..(14): um
  misc_feature (16)..(16): cm
  misc_feature (17)..(17): um
  misc_feature (20)..(20): um
augguauauguguugcugau

SEQ ID NO: 138 - RNA, 20 nt, Artificial Sequence
  synthesized siRNA antisense sequence
  misc_feature (3)..(3): cm
  misc_feature (6)..(6): cm
  misc_feature (9)..(9): cm
  misc_feature (11)..(11): cm
  misc_feature (13)..(13): um
  misc_feature (15)..(15): um
  misc_feature (18)..(18): cm
  misc_feature (19)..(20): um
aucagcaacacauauaccuu

SEQ ID NO: 139 - RNA, 19 nt, Artificial Sequence
  synthesized siRNA sense sequence
  misc_feature (1)..(1): um
  misc_feature (4)..(4): um
  misc_feature (6)..(6): um
  misc_feature (8)..(8): um
  misc_feature (10)..(10): um
  misc_feature (12)..(13): um
  misc_feature (15)..(15): cm
  misc_feature (16)..(16): um
  misc_feature (19)..(19): um
ugguauauguguugcugau

SEQ ID NO: 140 - RNA, 23 nt, Artificial Sequence
  synthesized siRNA antisense sequence
  misc_feature (3)..(3): cm
  misc_feature (6)..(6): cm
  misc_feature (9)..(9): cm
  misc_feature (11)..(11): cm
  misc_feature (13)..(13): um
  misc_feature (15)..(15): um
  misc_feature (18)..(18): cm
  misc_feature (20)..(23): um
aucagcaacacauauaccauuuu

SEQ ID NO: 141 - RNA, 19 nt, Artificial Sequence
  synthesized siRNA sense sequence
  misc_feature (1)..(1): um
  misc_feature (4)..(4): um
  misc_feature (6)..(6): um
  misc_feature (8)..(8): um
  misc_feature (10)..(10): um
  misc_feature (12)..(13): um
  misc_feature (16)..(16): um
  misc_feature (19)..(19): um
ugguauauguguugcugau

SEQ ID NO: 142 - RNA, 23 nt, Artificial Sequence
  synthesized siRNA antisense sequence
  misc_feature (3)..(3): cm
  misc_feature (6)..(6): cm
  misc_feature (9)..(9): cm
  misc_feature (11)..(11): cm
  misc_feature (13)..(13): um
  misc_feature (15)..(15): um
  misc_feature (18)..(18): cm
  misc_feature (20)..(23): um
aucagcaacacauauaccauuuu

SEQ ID NO: 143 - RNA, 19 nt, Artificial Sequence
  synthesized siRNA sense sequence
  misc_feature (1)..(1): um
  misc_feature (4)..(4): um
  misc_feature (6)..(6): um
  misc_feature (8)..(8): um
  misc_feature (10)..(10): um
  misc_feature (12)..(13): um
  misc_feature (16)..(16): um
  misc_feature (19)..(19): um
ugguauauguguugcugau

SEQ ID NO: 144 - RNA, 23 nt, Artificial Sequence
  synthesized siRNA antisense sequence
  misc_feature (3)..(3): cm
  misc_feature (6)..(6): cm
  misc_feature (9)..(9): cm
  misc_feature (11)..(11): cm
  misc_feature (13)..(13): um
  misc_feature (15)..(15): um
  misc_feature (18)..(18): cm
  misc_feature (20)..(21): um
  misc_feature (22)..(23): 2'-o-methyladenosine
aucagcaacacauauaccauuaa

SEQ ID NO: 145 - RNA, 19 nt, Artificial Sequence
  synthesized siRNA sense sequence
  misc_feature (1)..(1): um
  misc_feature (4)..(4): um
  misc_feature (6)..(6): um
  misc_feature (8)..(8): um
  misc_feature (10)..(10): um
  misc_feature (12)..(13): um
  misc_feature (16)..(16): um
  misc_feature (19)..(19): um
ugguauauguguugcugau

SEQ ID NO: 146 - RNA, 23 nt, Artificial Sequence
  synthesized siRNA antisense sequence
  misc_feature (3)..(3): cm
  misc_feature (6)..(6): cm
  misc_feature (9)..(9): cm
  misc_feature (11)..(11): cm
  misc_feature (13)..(13): um
  misc_feature (15)..(15): um
  misc_feature (18)..(18): cm
  misc_feature (20)..(21): um
  misc_feature (21)..(23): phosphorothioate bond
  misc_feature (22)..(23): 2'-o-methyladenosine
aucagcaacacauauaccauuaa

SEQ ID NO: 147 - RNA, 19 nt, Artificial Sequence
  synthesized siRNA sense sequence
  misc_feature (1)..(1): um
  misc_feature (4)..(4): um
  misc_feature (6)..(6): um
  misc_feature (8)..(8): um
  misc_feature (10)..(10): um
  misc_feature (12)..(13): um
  misc_feature (16)..(16): um
  misc_feature (19)..(19): um
ugguauauguguugcugau

SEQ ID NO: 148 - RNA, 23 nt, Artificial Sequence
  synthesized siRNA antisense sequence
  misc_feature (3)..(3): cm
  misc_feature (6)..(6): cm
  misc_feature (9)..(9): cm
  misc_feature (11)..(11): cm
  misc_feature (13)..(13): um
  misc_feature (15)..(15): um
  misc_feature (18)..(18): cm
  misc_feature (19)..(21): phosphorothioate bond
  misc_feature (20)..(21): um
  misc_feature (22)..(23): 2'-o-methyladenosine
aucagcaacacauauaccauuaa

SEQ ID NO: 149 - RNA, 19 nt, Artificial Sequence
  synthesized siRNA sense sequence
  misc_feature (1)..(1): um
  misc_feature (4)..(4): um
  misc_feature (6)..(6): um
  misc_feature (8)..(8): um
  misc_feature (10)..(10): um
  misc_feature (12)..(13): um
  misc_feature (16)..(16): um
  misc_feature (19)..(19): um
ugguauauguguugcugau

SEQ ID NO: 150 - RNA, 23 nt, Artificial Sequence
  synthesized siRNA antisense sequence
  misc_feature (1)..(1): 2'-o-methyladenosine
  misc_feature (1)..(2): phosphorothioate bond
  misc_feature (3)..(3): cm
  misc_feature (6)..(6): cm
  misc_feature (9)..(9): cm
  misc_feature (11)..(11): cm
  misc_feature (13)..(13): um
  misc_feature (15)..(15): um
  misc_feature (18)..(18): cm
  misc_feature (19)..(21): phosphorothioate bond
  misc_feature (20)..(21): um
  misc_feature (22)..(23): 2'-o-methyladenosine
aucagcaacacauauaccauuaa

SEQ ID NO: 151 - RNA, 19 nt, Artificial Sequence
  synthesized siRNA sense sequence
  misc_feature (1)..(1): um
  misc_feature (4)..(4): um
  misc_feature (6)..(6): um
  misc_feature (8)..(8): um
  misc_feature (10)..(10): um
  misc_feature (12)..(13): um
  misc_feature (16)..(16): um
  misc_feature (19)..(19): um
ugguauauguguugcugau

SEQ ID NO: 152 - RNA, 23 nt, Artificial Sequence
  synthesized siRNA antisense sequence
  misc_feature (1)..(1): 2'-o-methyladenosine
  misc_feature (3)..(3): cm
  misc_feature (6)..(6): cm
  misc_feature (9)..(9): cm
  misc_feature (11)..(11): cm
  misc_feature (13)..(13): um
  misc_feature (15)..(15): um
  misc_feature (18)..(18): cm
  misc_feature (20)..(23): um
aucagcaacacauauaccauuuu

SEQ ID NO: 153 - RNA, 19 nt, Artificial Sequence
  synthesized siRNA sense sequence
  misc_feature (1)..(1): um
  misc_feature (1)..(2): phosphorothioate bond
  misc_feature (4)..(4): um
  misc_feature (6)..(6): um
  misc_feature (8)..(8): um
  misc_feature (10)..(10): um
  misc_feature (12)..(13): um
  misc_feature (16)..(16): um
  misc_feature (19)..(19): um
ugguauauguguugcugau

SEQ ID NO: 154 - RNA, 23 nt, Artificial Sequence
  synthesized siRNA antisense sequence
  misc_feature (3)..(3): cm
  misc_feature (6)..(6): cm
  misc_feature (9)..(9): cm
  misc_feature (11)..(11): cm
  misc_feature (13)..(13): um
  misc_feature (15)..(15): um
  misc_feature (18)..(18): cm
  misc_feature (19)..(21): phosphorothioate bond
  misc_feature (20)..(21): um
  misc_feature (22)..(23): 2'-o-methyladenosine
aucagcaacacauauaccauuaa

SEQ ID NO: 155 - RNA, 21 nt, Artificial Sequence
  synthesized siRNA sense sequence
  misc_feature (2)..(2): um
  misc_feature (5)..(5): cm
  misc_feature (6)..(6): um
  misc_feature (7)..(7): cm
  misc_feature (9)..(9): cm
  misc_feature (10)..(10): um
  misc_feature (12)..(12): um
  misc_feature (15)..(16): um
  misc_feature (18)..(18): cm
  misc_feature (19)..(19): um
  misc_feature (20)..(21): n=deoxythymidine
  misc_feature (20)..(21): phosphorothioate bond
auaacucacuauaauuacunn

SEQ ID NO: 156 - RNA, 21 nt, Artificial Sequence
  synthesized siRNA antisense sequence
  misc_feature (3)..(3): um
  misc_feature (7)..(7): um
  misc_feature (9)..(9): um
  misc_feature (17)..(17): um
  misc_feature (20)..(21): n=deoxythymidine
  misc_feature (20)..(21): phosphorothioate bond
aguaauuauagugaguuaunn

SEQ ID NO: 157 - RNA, 19 nt, Artificial Sequence
  synthesized siRNA sense sequence
  misc_feature (2)..(2): um
  misc_feature (5)..(5): cm
  misc_feature (6)..(6): um
  misc_feature (7)..(7): cm
  misc_feature (9)..(9): cm
  misc_feature (10)..(10): um
  misc_feature (12)..(12): um
  misc_feature (15)..(16): um
  misc_feature (18)..(18): cm
  misc_feature (19)..(19): um
auaacucacuauaauuacu

SEQ ID NO: 158 - RNA, 19 nt, Artificial Sequence
  synthesized siRNA antisense sequence
  misc_feature (3)..(3): um
  misc_feature (7)..(7): um
  misc_feature (9)..(9): um
  misc_feature (17)..(17): um
aguaauuauagugaguuau

SEQ ID NO: 159 - RNA, 21 nt, Artificial Sequence
  synthesized siRNA sense sequence
  misc_feature (1)..(1): um
  misc_feature (4)..(4): um
  misc_feature (6)..(6): um
  misc_feature (8)..(8): um
  misc_feature (10)..(10): um
  misc_feature (12)..(13): um
  misc_feature (15)..(15): cm
  misc_feature (16)..(16): um
  misc_feature (19)..(21): um
ugguauauguguugcugauuu

SEQ ID NO: 160 - RNA, 21 nt, Artificial Sequence
  synthesized siRNA antisense sequence
  misc_feature (3)..(3): cm
  misc_feature (6)..(6): cm
  misc_feature (9)..(9): cm
  misc_feature (11)..(11): cm
  misc_feature (13)..(13): um
  misc_feature (15)..(15): um
  misc_feature (18)..(18): cm
  misc_feature (20)..(21): um
aucagcaacacauauaccauu

SEQ ID NO: 161 - RNA, 21 nt, Artificial Sequence
  synthesized siRNA sense sequence
  misc_feature (4)..(4): cm
  misc_feature (10)..(10): um
  misc_feature (12)..(13): um
  misc_feature (14)..(14): cm
  misc_feature (20)..(21): um
aggcaaagguguucaaagauu

SEQ ID NO: 162 - RNA, 21 nt, Artificial Sequence
  synthesized siRNA antisense sequence
  misc_feature (9)..(9): cm
  misc_feature (20)..(21): um
ucuuugaacaccuuugccuuu

SEQ ID NO: 163 - RNA, 21 nt, Artificial Sequence
  synthesized siRNA sense sequence
  misc_feature (9)..(9): cm
  misc_feature (10)..(10): um
  misc_feature (12)..(14): um
  misc_feature (16)..(16): cm
  misc_feature (19)..(19): cm
  misc_feature (20)..(21): um
gaaaggaacuguuuacaacuu

SEQ ID NO: 164 - RNA, 21 nt, Artificial Sequence
  synthesized siRNA antisense sequence
  misc_feature (5)..(5): um
  misc_feature (9)..(9): cm
  misc_feature (20)..(21): um
guuguaaacaguuccuuucuu

SEQ ID NO: 165 - RNA, 21 nt, Artificial Sequence
  synthesized siRNA sense sequence
  misc_feature (2)..(2): cm
  misc_feature (3)..(3): um
  misc_feature (6)..(6): um
  misc_feature (8)..(8): um
  misc_feature (10)..(10): um
  misc_feature (12)..(12): um
  misc_feature (14)..(15): um
  misc_feature (17)..(17): cm
  misc_feature (18)..(18): um
  misc_feature (20)..(21): n=deoxythymidine
  misc_feature (20)..(21): phosphorothioate bond
acugguauauguguugcugnn

SEQ ID NO: 166 - RNA, 21 nt, Artificial Sequence
  synthesized siRNA antisense sequence
  misc_feature (1)..(1): cm
  misc_feature (4)..(4): cm
  misc_feature (7)..(7): cm
  misc_feature (9)..(9): cm
  misc_feature (11)..(11): um
  misc_feature (13)..(13): um
  misc_feature (16)..(16): cm
  misc_feature (20)..(21): n=deoxythymidine
  misc_feature (20)..(21): phosphorothioate bond
cagcaacacauauaccagunn

SEQ ID NO: 167 - RNA, 21 nt, Artificial Sequence
  synthesized siRNA sense sequence
  misc_feature (1)..(1): cm
  misc_feature (2)..(2): um
  misc_feature (5)..(5): um
  misc_feature (7)..(7): um
  misc_feature (9)..(9): um
  misc_feature (11)..(11): um
  misc_feature (13)..(14): um
  misc_feature (16)..(16): cm
  misc_feature (17)..(17): um
  misc_feature (20)..(21): n=deoxythymidine
  misc_feature (20)..(21): phosphorothioate bond
cugguauauguguugcugann

SEQ ID NO: 168 - RNA, 21 nt, Artificial Sequence
  synthesized siRNA antisense sequence
  misc_feature (2)..(2): cm
  misc_feature (5)..(5): cm
  misc_feature (8)..(8): cm
  misc_feature (10)..(10): cm
  misc_feature (12)..(12): um
  misc_feature (14)..(14): um
  misc_feature (17)..(17): cm
  misc_feature (20)..(21): n=deoxythymidine
  misc_feature (20)..(21): phosphorothioate bond
ucagcaacacauauaccagnn

SEQ ID NO: 169 - RNA, 21 nt, Artificial Sequence
  synthesized siRNA sense sequence
  misc_feature (3)..(3): um
  misc_feature (5)..(5): um
  misc_feature (7)..(7): um
  misc_feature (9)..(9): um
  misc_feature (11)..(12): um
  misc_feature (14)..(14): cm
  misc_feature (15)..(15): um
  misc_feature (18)..(18): um
  misc_feature (20)..(21): n=deoxythymidine
  misc_feature (20)..(21): phosphorothioate bond
gguauauguguugcugauann

SEQ ID NO: 170 - RNA, 21 nt, Artificial Sequence
  synthesized siRNA antisense sequence
  misc_feature (1)..(1): um
  misc_feature (4)..(4): cm
  misc_feature (7)..(7): cm
  misc_feature (10)..(10): cm
  misc_feature (12)..(12): cm
  misc_feature (14)..(14): um
  misc_feature (16)..(16): um
  misc_feature (20)..(21): n=deoxythymidine
  misc_feature (20)..(21): phosphorothioate bond
uaucagcaacacauauaccnn

SEQ ID NO: 171 - RNA, 21 nt, Artificial Sequence
  synthesized siRNA sense sequence
  misc_feature (2)..(2): um
  misc_feature (4)..(4): um
  misc_feature (6)..(6): um
  misc_feature (8)..(8): um
  misc_feature (10)..(11): um
  misc_feature (13)..(13): cm
  misc_feature (14)..(14): um
  misc_feature (17)..(17): um
  misc_feature (19)..(19): cm
  misc_feature (20)..(21): n=deoxythymidine
  misc_feature (20)..(21): phosphorothioate bond
guauauguguugcugauacnn

SEQ ID NO: 172 - RNA, 21 nt, Artificial Sequence
  synthesized siRNA antisense sequence
  misc_feature (2)..(2): um
  misc_feature (5)..(5): cm
  misc_feature (8)..(8): cm
  misc_feature (11)..(11): cm
  misc_feature (13)..(13): cm
  misc_feature (15)..(15): um
  misc_feature (17)..(17): um
  misc_feature (20)..(21): n=deoxythymidine
  misc_feature (20)..(21): phosphorothioate bond
guaucagcaacacauauacnn